European Patent Specification EP 3 967 712 B1, published January 3, 2024. Title: Recombinant Monoclonal Antibodies And Corresponding Antigens for Colon and Pancreatic Cancer. Applicant: Precision Biologics, Inc. The sequence listing filed with the application follows.

SEQUENCE LISTING (29 sequences)

SEQ ID NO: 1 - protein, 11 aa, Mus musculus
GASENIYGALN

SEQ ID NO: 2 - protein, 7 aa, Mus musculus
GASNLAD

SEQ ID NO: 3 - protein, 9 aa, Mus musculus
QNVLSSPYT

SEQ ID NO: 4 - protein, 11 aa, Homo sapiens
QASENIYGALN

SEQ ID NO: 5 - protein, 7 aa, Homo sapiens
GASNLAT

SEQ ID NO: 6 - protein, 9 aa, Homo sapiens
QQVLSSPYT

SEQ ID NO: 7 - protein, 10 aa, Mus musculus
GYTFTDYAMH

SEQ ID NO: 8 - protein, 17 aa, Mus musculus
LISTYSGDTKYNQNFKG

SEQ ID NO: 9 - protein, 12 aa, Mus musculus
GDYSGSRYWFAY

SEQ ID NO: 10 - protein, 17 aa, Homo sapiens
LISTYSGDTKYNQNFQG

SEQ ID NO: 11 - protein, 12 aa, Homo sapiens
GDYSGSRYWFAY

SEQ ID NO: 12 - DNA, 965 bp, Mus musculus
gcggggcagcctcacacagaacacacacagatatgggtgtacccactcagctcctgttgctgtggcttacagtcgtagttgtcagatgtgacatccagatgactcagtctccagcttcactgtctgcatctgtgggagaaactgtcaccatcacatgtggagcaagtgagaatatttacggtgctttaaattggtatcagcggaaacagggaaaatctcctcagctcctgatttatggcgcaagtaatttggcagatggcatgtcatcgaggttcagtggcagtggatctggtagacagtattctctcaagatcagtagcctgcatcctgacgatgttgcaacgtattactgtcaaaatgtattaagtagtccgtacacgttcggaggggggaccaagctggaaataaaacgggctgatgctgcaccaactgtatccatcttcccaccatccagtgagcagttaacatctggaggtgcctcagtcgtgtgcttcttgaacaacttctaccccaaagacatcaatgtcaagtggaagattgatggcagtgaacgacaaaatggcgtcctgaacagttggactgatcaggacagcaaagacagcacctacagcatgagcagcaccctcacgttgaccaaggacgagtatgaacgacataacagctatacctgtgaggccactcacaagacaccaacttcacccattgtcaagagcttcaacaggaatgagtgttagagacaaaggtcctgagacgccaccaccagctccccagctccatcctatcttcccttctaaggtcttggaggcttccccacaagcgacctaccactgttgcggtgctccaaacctcctccccacctccttctcctcctcctccctttccttggcttttatcatgctaatatttgcagaaaatattcaataaagtgagtctttgcacaaaaaaaaaaaaaaaaaaaaaaaaaa

SEQ ID NO: 13 - DNA, 1575 bp, Mus musculus
acgcgggacacagtagtctctacagtcacaggagtacacaggacattgccatgggttggagctgtatcatcttctttctggtagcaacagctacaggtgtgcactcccaggtccagctgcagcagtctgggcctgaggtggtgaggcctggggtctcagtgaagatttcctgcaagggttccggctacacattcactgattatgctatgcactgggtgaagcagagtcatgcaaagagtctcgagtggattggacttattagtacttacagtggtgatacaaagtacaaccagaactttaagggcaaggccacaatgactgtagacaaatcctccaacacagcctatatggaacttgccagattgacatctgaggattctgccatctattactgtgcaagaggggattattccggtagtaggtactggtttgcttactggggccaagggactctggtcactgtctctgcagccaaaacgacacccccatctgtctatccactggcccctggatctgctgcccaaactaactccatggtgaccctgggatgcctggtcaagggctatttccctgagccagtgacagtgacctggaactctggatccctgtccagcggtgtgcacaccttcccagctgtcctgcagtctgacctctacactctgagcagctcagtgactgtcccctccagcacctggcccagcgagaccgtcacctgcaacgttgcccacccggccagcagcaccaaggtggacaagaaaattgtgcccagggattgtggttgtaagccttgcatatgtacagtcccagaagtatcatctgtcttcatcttccccccaaagcccaaggatgtgctcaccattactctgactcctaaggtcacgtgtgttgtggtagacatcagcaaggatgatcccgaggtccagttcagctggtttgtagatgatgtggaggtgcacacagctcagacgcaaccccgggaggagcagttcaacagcactttccgctcagtcagtgaacttcccatcatgcaccaggactggctcaatggcaaggagttcaaatgcagggtcaacagtgcagctttccctgcccccatcgagaaaaccatctccaaaaccaaaggcagaccgaaggctccacaggtgtacaccattccacctcccaaggagcagatggccaaggataaagtcagtctgacctgcatgataacagacttcttccctgaagacattactgtggagtggcagtggaatgggcagccagcggagaactacaagaacactcagcccatcatggacacagatggctcttacttcgtctacagcaagctcaatgtgcagaagagcaactgggaggcaggaaatactttcacctgctctgtgttacatgagggcctgcacaaccaccatactgagaagagcctctcccactctcctggtaaatgatcccagtgtccttggagccctctggccctacaggactttgacacctacctccacccctccctgtataaataaagcacccagcactgcctcgggaccctgcataaaaaaaaaaaaaaaaaaaaaaaaaaaa

SEQ ID NO: 14 - protein, 107 aa, Mus musculus
LMTQSPASLSASVGETVTITCGASENIYGALNWYQRKQGKSPQLLIYGASNLADGMSSRFSGSGSGRQYSLKISSLHPDDVATYYCQNVLSSPYTFGGGTKLEIKKG

SEQ ID NO: 15 - protein, 116 aa, Mus musculus
LEESGPEVVRPGVSVKISCKGSGYTFTDYAMHWVKQSHAKSLEWIGLISTYSGDTKYNQNFKGKATMTVDKSSNTAYMELARLTSEDSAIYYCARGDYSGSRYWFAYWGQGTTVTR

SEQ ID NO: 16 - protein, 107 aa, Mus musculus
DIQMTQSPASLSASVGETVTITCGASENIYGALNWYQRKQGKSPQLLIYGASNLADGMSSRFSGSGSGRQYSLKISSLHPDDVATYYCQNVLSSPYTFGGGTKLEIK

SEQ ID NO: 17 - protein, 107 aa, Artificial Sequence
  humanized mAb sequence
DIQMTQSPSSLSASVGDRVTITCGASENIYGALNWYQRKPGKSPKLLIYGASNLADGMPSRFSGSGSGRQYTLTISSLQPEDVATYYCQNVLSSPYTFGGGTKLEIK

SEQ ID NO: 18 - protein, 107 aa, Artificial Sequence; identical to SEQ ID NO: 17
  humanized mAb sequences

SEQ ID NO: 19 - protein, 107 aa, Artificial Sequence
  humanized mAb sequences
DIQMTQSPSSLSASVGDRVTITCQASENIYGALNWYQRKPGKSPKLLIYGASNLATGMPSRFSGSGSGTDYTFTISSLQPEDIATYYCQNVLSSPYTFGGGTKLEIK

SEQ ID NO: 20 - protein, 107 aa, Artificial Sequence
  humanized mAb sequence
DIQMTQSPSSLSASVGDRVTITCGASENIYGALNWYQRKPGKSPKLLIYGASNLATGMPSRFSGSGSGRQYTFTISSLQPEDIATYYCQQVLSSPYTFGGGTKLEIK

SEQ ID NO: 21 - protein, 107 aa, Artificial Sequence
  humanized mAb sequence
DIQMTQSPSSLSASVGDRVTITCGASENIYGALNWYQRKPGKSPNLLIYGASNLADGMPSRFSGSGSGRQYTLTISSLQPEDVATYYCQNVLSSPYTFGGGTKLEIK

SEQ ID NO: 22 - protein, 121 aa, Mus musculus
QVQLQQSGPEVVRPGVSVKISCKGSGYTFTDYAMHWVKQSHAKSLEWIGLISTYSGDTKYNQNFKGKATMTVDKSSNTAYMELARLTSEDSAIYYCARGDYSGSRYWFAYWGQGTLVTVSA

SEQ ID NO: 23 - protein, 121 aa, Artificial Sequence
  humanized mAb sequence
QVQLVQSGAEVKKPGASVKVSCKGSGYTFTDYAMHWVRQAPGQRLEWIGLISTYSGDTKYNQNFKGKATMTVDKSASTAYMELSSLRSEDTAVYYCARGDYSGSRYWFAYWGQGTLVTVSS

SEQ ID NO: 24 - protein, 121 aa, Artificial Sequence
  humanized mAb sequence
QVQLVQSGAEVKKPGASVKVSCKGSGYTFTDYAMHWVRQAPGQGLEWIGLISTYSGDTKYNQNFKGKATMTVDTSISTAYMELSRLRSDDTAIYYCARGDYSGSRYWFAYWGQGTLVTVSS

SEQ ID NO: 25 - protein, 121 aa, Artificial Sequence
  humanized mAb sequences
QVQLVQSGAEVKKPGASVKVSCKASGYTFTDYAMHWVRQAPGQRLEWMGLISTYSGDTKYSQKFQGRVTMTVDKSASTAYMELSSLRSEDTAVYYCARGDYSGSRYWFAYWGQGTLVTVSS

SEQ ID NO: 26 - protein, 121 aa, Artificial Sequence
  humanized mAb sequence
QVQLVQSGAEVKKPGASVKVSCKASGYTFTDYAMHWVRQAPGQRLEWIGLISTYSGDTKYNQKFQGKATMTVDKSASTAYMELSSLRSEDTAVYYCARGDYSGSRYWFAYWGQGTLVTVSS

SEQ ID NO: 27 - protein, 121 aa, Artificial Sequence
  humanized mAb sequence
QVQLVQSGAEVKKPGASVKVSCKGSGYTFTDYAMHWVRQVHAQGLEWIGLISTYSGDTKYNQNFKGKATMTVDKSTSTAYMELSSLRSEDTAVYYCARGDYSGSRYWFAYWGQGTLVTVSS

SEQ ID NO: 28 - protein, 470 aa, Artificial Sequence
  Optimized humanized mAb sequence
MGWSCIIFFLVATATGVHSQVQLVQSGAEVKKPGASVKVSCKASGYTFTDYAMHWVRQAPGQRLEWMGLISTYSGDTKYNQNFQGRVTMTVDKSASTAYMELSSLRSEDTAVYYCARGDYSGSRYWFAYWGQGTLVTVSSASTKGPSVFPLAPSSKSTSGGTAALGCLVKDYFPEPVTVSWNSGALTSGVHTFPAVLQSSGLYSLSSVVTVPSSSLGTQTYICNVNHKPSNTKVDKKVEPKSCDKTHTCPPCPAPELLGGPSVFLFPPKPKDTLMISRTPEVTCVVVDVSHEDPEVKFNWYVDGVEVHNAKTKPREEQYNSTYRVVSVLTVLHQDWLNGKEYKCKVSNKALPAPIEKTISKAKGQPREPQVYTLPPSRDELTKNQVSLTCLVKGFYPSDIAVEWESNGQPENNYKTTPPVLDSDGSFFLYSKLTVDKSRWQQGNVFSCSVMHEALHNHYTQKSLSLSPGK

SEQ ID NO: 29 - protein, 233 aa, Artificial Sequence
  optimized, humanized mAb sequence
MGVPTQLLLLWLTVVVVRCDIQMTQSPSSLSASVGDRVTITCQASENIYGALNWYQRKPGKSPKLLIYGASNLATGMPSRFSGSGSGTDYTFTISSLQPEDIATYYCQQVLSSPYTFGGGTKLEIKRTVAAPSVFIFPPSDEQLKSGTASVVCLLNNFYPREAKVQWKVDNALQSGNSQESVTEQDSKDSTYSLSSTLTLSKADYEKHKVYACEVTHQGLSSPVTKSFNRGEC